European Patent Application EP 4 183 802 A1, published May 24, 2023. Title: ANTI-ANG-2 ANTIBODY AND USE THEREOF. Applicant: INNOVENT BIOLOGICS (SUZHOU) CO., LTD. The sequence listing filed with the application follows.

SEQUENCE LISTING (60 sequences)

SEQ ID NO: 1 - protein, 10 aa, artificial sequence
  synthetic
GFTFSNYWMN

SEQ ID NO: 2 - protein, 19 aa, artificial sequence
  synthetic
EIRLKSNNYATHYAESVKG

SEQ ID NO: 3 - protein, 6 aa, artificial sequence
  synthetic
TAPFAY

SEQ ID NO: 4 - protein, 11 aa, artificial sequence
  synthetic
KASQDVGTDVA

SEQ ID NO: 5 - protein, 7 aa, artificial sequence
  synthetic
WASTRHT

SEQ ID NO: 6 - protein, 9 aa, artificial sequence
  synthetic
QQYSSYPLT

SEQ ID NO: 7 - protein, 10 aa, artificial sequence
  synthetic
GFTFRAAWMN

SEQ ID NO: 8 - protein, 19 aa, artificial sequence
  synthetic
EIRLKSNHYETHYAESVKG

SEQ ID NO: 9 - protein, 6 aa, artificial sequence
  synthetic
TQPGAY

SEQ ID NO: 10 - protein, 11 aa, artificial sequence
  synthetic
KASQYVFTDVA

SEQ ID NO: 11 - protein, 7 aa, artificial sequence
  synthetic
WASTRWT

SEQ ID NO: 12 - protein, 9 aa, artificial sequence
  synthetic
QQTSSYPLT

SEQ ID NO: 13 - protein, 10 aa, artificial sequence
  synthetic
GFTFQNYWAN

SEQ ID NO: 14 - protein, 19 aa, artificial sequence
  synthetic
EIRLKSNNYATHYAESVKG

SEQ ID NO: 15 - protein, 6 aa, artificial sequence
  synthetic
TTPAAY

SEQ ID NO: 16 - protein, 11 aa, artificial sequence
  synthetic
KASQDVWTDVA

SEQ ID NO: 17 - protein, 7 aa, artificial sequence
  synthetic
WGSTRWT

SEQ ID NO: 18 - protein, 9 aa, artificial sequence
  synthetic
QQTNIYPLT

SEQ ID NO: 19 - protein, 117 aa, artificial sequence
  synthetic
EVKLEESGGGLVQPGGSMKLSCVASGFTFSNYWMNWVRQSPEKGLEWVAEIRLKSNNYATHYAESVKGRFTISRDVSKSSVYLQMNNLRTEDTGIYYCTDTAPFAYWGQGTLVTVSA

SEQ ID NO: 20 - protein, 107 aa, artificial sequence
  synthetic
DIVMTQSHKFMSTSVGDRVSITCKASQDVGTDVAWYQQKPGQSPKLLIYWASTRHTGVPDRFTGSGSGTDFTLTISNVQSEDLSDYFCQQYSSYPLTFGGGTKLEIK

SEQ ID NO: 21 - protein, 117 aa, artificial sequence
  synthetic
EVMLVESGGGLVQPGGSMKLSCVASGFTFSNYWMNWVRQSPEKGLEWVAEIRLKSNNYATHYAESVKGRFTISRDVSKSGVYLQMNNLRTEDTGIYYCTDTAPFAYWGQGTLVTVSA

SEQ ID NO: 22 - protein, 107 aa, artificial sequence
  synthetic
DIVMTQSHKFLSTSVGARVSITCKASQDVGTDVAWYQQKPGQSPKLLIYWASTRHTGVPDRFTGSGSGTDFTLTISNVQSEDLSDYFCQQYSSYPLTFGGGTKLEIK

SEQ ID NO: 23 - protein, 117 aa, artificial sequence; identical to SEQ ID NO: 21
  synthetic

SEQ ID NO: 24 - protein, 107 aa, artificial sequence
  synthetic
DIVMTQTPKFLSTSVGARVSITCKASQDVGTDVAWYQQKPGQSPKLLIYWASTRHTGVPDRFTGSGSGTDFTLTISNVQSEDLSDYFCQQYSSYPLTFGGGTKLEIK

SEQ ID NO: 25 - protein, 117 aa, artificial sequence
  synthetic
EVQLVESGGGLVKPGGSLRLSCAASGFTFSNYWMNWVRQAPGKGLEWVAEIRLKSNNYATHYAESVKGRFTISRDVSKNTVYLQMNSLKTEDTAVYYCTDTAPFAYWGQGTLVTVSS

SEQ ID NO: 26 - protein, 107 aa, artificial sequence
  synthetic
DIQMTQSPSSLSASVGDRVTITCKASQDVGTDVAWYQQKPGKAPKLLIYWASTRHTGVPSRFSGSGSGTDFTLTISSLQPEDFATYYCQQYSSYPLTFGGGTKVEIK

SEQ ID NO: 27 - protein, 117 aa, artificial sequence
  synthetic
EVQLVESGGGLVKPGGSLRLSCAASGFTFRAAWMNWVRQAPGKGLEWVAEIRLKSNHYETHYAESVKGRFTISRDVSKNTVYLQMNSLKTEDTAVYYCTDTQPGAYWGQGTLVTVSS

SEQ ID NO: 28 - protein, 107 aa, artificial sequence
  synthetic
DIQMTQSPSSLSASVGDRVTITCKASQYVFTDVAWYQQKPGKAPKLLIYWASTRWTGVPSRFSGSGSGTDFTLTISSLQPEDFATYYCQQTSSYPLTFGGGTKVEIK

SEQ ID NO: 29 - protein, 117 aa, artificial sequence
  synthetic
EVQLVESGGGLVKPGGSLRLSCAASGFTFQNYWANWVRQAPGKGLEWVAEIRLKSNNYATHYAESVKGRFTISRDVSKNTVYLQMNSLKTEDTAVYYCTDTTPAAYWGQGTLVTVSS

SEQ ID NO: 30 - protein, 107 aa, artificial sequence
  synthetic
DIQMTQSPSSLSASVGDRVTITCKASQDVWTDVAWYQQKPGKAPKLLIYWGSTRWTGVPSRFSGSGSGTDFTLTISSLQPEDFATYYCQQTNIYPLTFGGGTKVEIK

SEQ ID NO: 31 - protein, 447 aa, artificial sequence
  synthetic
EVKLEESGGGLVQPGGSMKLSCVASGFTFSNYWMNWVRQSPEKGLEWVAEIRLKSNNYATHYAESVKGRFTISRDVSKSSVYLQMNNLRTEDTGIYYCTDTAPFAYWGQGTLVTVSAASTKGPSVFPLAPSSKSTSGGTAALGCLVKDYFPEPVTVSWNSGALTSGVHTFPAVLQSSGLYSLSSVVTVPSSSLGTQTYICNVNHKPSNTKVDKKAEPKSCDKTHTCPPCPAPELLGGPSVFLFPPKPKDTLMISRTPEVTCVVVDVSHEDPEVKFNWYVDGVEVHNAKTKPREEQYNSTYRVVSVLTVLHQDWLNGKEYKCKVSNKALPAPIEKTISKAKGQPREPQVYTLPPSRDELTKNQVSLTCLVKGFYPSDIAVEWESNGQPENNYKTTPPVLDSDGSFFLYSKLTVDKSRWQQGNVFSCSVMHEALHNHYTQKSLSLSPGK

SEQ ID NO: 32 - protein, 214 aa, artificial sequence
  synthetic
DIVMTQSHKFMSTSVGDRVSITCKASQDVGTDVAWYQQKPGQSPKLLIYWASTRHTGVPDRFTGSGSGTDFTLTISNVQSEDLSDYFCQQYSSYPLTFGGGTKLEIKRTVAAPSVFIFPPSDEQLKSGTASVVCLLNNFYPREAKVQWKVDNALQSGNSQESVTEQDSKDSTYSLSSTLTLSKADYEKHKVYACEVTHQGLSSPVTKSFNRGEC

SEQ ID NO: 33 - protein, 447 aa, artificial sequence
  synthetic
EVMLVESGGGLVQPGGSMKLSCVASGFTFSNYWMNWVRQSPEKGLEWVAEIRLKSNNYATHYAESVKGRFTISRDVSKSGVYLQMNNLRTEDTGIYYCTDTAPFAYWGQGTLVTVSAASTKGPSVFPLAPSSKSTSGGTAALGCLVKDYFPEPVTVSWNSGALTSGVHTFPAVLQSSGLYSLSSVVTVPSSSLGTQTYICNVNHKPSNTKVDKKAEPKSCDKTHTCPPCPAPELLGGPSVFLFPPKPKDTLMISRTPEVTCVVVDVSHEDPEVKFNWYVDGVEVHNAKTKPREEQYNSTYRVVSVLTVLHQDWLNGKEYKCKVSNKALPAPIEKTISKAKGQPREPQVYTLPPSRDELTKNQVSLTCLVKGFYPSDIAVEWESNGQPENNYKTTPPVLDSDGSFFLYSKLTVDKSRWQQGNVFSCSVMHEALHNHYTQKSLSLSPGK

SEQ ID NO: 34 - protein, 214 aa, artificial sequence
  synthetic
DIVMTQSHKFLSTSVGARVSITCKASQDVGTDVAWYQQKPGQSPKLLIYWASTRHTGVPDRFTGSGSGTDFTLTISNVQSEDLSDYFCQQYSSYPLTFGGGTKLEIKRTVAAPSVFIFPPSDEQLKSGTASVVCLLNNFYPREAKVQWKVDNALQSGNSQESVTEQDSKDSTYSLSSTLTLSKADYEKHKVYACEVTHQGLSSPVTKSFNRGEC

SEQ ID NO: 35 - protein, 447 aa, artificial sequence; identical to SEQ ID NO: 33
  synthetic

SEQ ID NO: 36 - protein, 214 aa, artificial sequence
  synthetic
DIVMTQTPKFLSTSVGARVSITCKASQDVGTDVAWYQQKPGQSPKLLIYWASTRHTGVPDRFTGSGSGTDFTLTISNVQSEDLSDYFCQQYSSYPLTFGGGTKLEIKRTVAAPSVFIFPPSDEQLKSGTASVVCLLNNFYPREAKVQWKVDNALQSGNSQESVTEQDSKDSTYSLSSTLTLSKADYEKHKVYACEVTHQGLSSPVTKSFNRGEC

SEQ ID NO: 37 - protein, 447 aa, artificial sequence
  synthetic
EVQLVESGGGLVKPGGSLRLSCAASGFTFSNYWMNWVRQAPGKGLEWVAEIRLKSNNYATHYAESVKGRFTISRDVSKNTVYLQMNSLKTEDTAVYYCTDTAPFAYWGQGTLVTVSSASTKGPSVFPLAPSSKSTSGGTAALGCLVKDYFPEPVTVSWNSGALTSGVHTFPAVLQSSGLYSLSSVVTVPSSSLGTQTYICNVNHKPSNTKVDKKAEPKSCDKTHTCPPCPAPELLGGPSVFLFPPKPKDTLMISRTPEVTCVVVDVSHEDPEVKFNWYVDGVEVHNAKTKPREEQYNSTYRVVSVLTVLHQDWLNGKEYKCKVSNKALPAPIEKTISKAKGQPREPQVYTLPPSRDELTKNQVSLTCLVKGFYPSDIAVEWESNGQPENNYKTTPPVLDSDGSFFLYSKLTVDKSRWQQGNVFSCSVMHEALHNHYTQKSLSLSPGK

SEQ ID NO: 38 - protein, 214 aa, artificial sequence
  synthetic
DIQMTQSPSSLSASVGDRVTITCKASQDVGTDVAWYQQKPGKAPKLLIYWASTRHTGVPSRFSGSGSGTDFTLTISSLQPEDFATYYCQQYSSYPLTFGGGTKVEIKRTVAAPSVFIFPPSDEQLKSGTASVVCLLNNFYPREAKVQWKVDNALQSGNSQESVTEQDSKDSTYSLSSTLTLSKADYEKHKVYACEVTHQGLSSPVTKSFNRGEC

SEQ ID NO: 39 - protein, 447 aa, artificial sequence
  synthetic
EVQLVESGGGLVKPGGSLRLSCAASGFTFRAAWMNWVRQAPGKGLEWVAEIRLKSNHYETHYAESVKGRFTISRDVSKNTVYLQMNSLKTEDTAVYYCTDTQPGAYWGQGTLVTVSSASTKGPSVFPLAPSSKSTSGGTAALGCLVKDYFPEPVTVSWNSGALTSGVHTFPAVLQSSGLYSLSSVVTVPSSSLGTQTYICNVNHKPSNTKVDKKAEPKSCDKTHTCPPCPAPELLGGPSVFLFPPKPKDTLMISRTPEVTCVVVDVSHEDPEVKFNWYVDGVEVHNAKTKPREEQYNSTYRVVSVLTVLHQDWLNGKEYKCKVSNKALPAPIEKTISKAKGQPREPQVYTLPPSRDELTKNQVSLTCLVKGFYPSDIAVEWESNGQPENNYKTTPPVLDSDGSFFLYSKLTVDKSRWQQGNVFSCSVMHEALHNHYTQKSLSLSPGK

SEQ ID NO: 40 - protein, 214 aa, artificial sequence
  synthetic
DIQMTQSPSSLSASVGDRVTITCKASQYVFTDVAWYQQKPGKAPKLLIYWASTRWTGVPSRFSGSGSGTDFTLTISSLQPEDFATYYCQQTSSYPLTFGGGTKVEIKRTVAAPSVFIFPPSDEQLKSGTASVVCLLNNFYPREAKVQWKVDNALQSGNSQESVTEQDSKDSTYSLSSTLTLSKADYEKHKVYACEVTHQGLSSPVTKSFNRGEC

SEQ ID NO: 41 - protein, 447 aa, artificial sequence
  synthetic
EVQLVESGGGLVKPGGSLRLSCAASGFTFQNYWANWVRQAPGKGLEWVAEIRLKSNNYATHYAESVKGRFTISRDVSKNTVYLQMNSLKTEDTAVYYCTDTTPAAYWGQGTLVTVSSASTKGPSVFPLAPSSKSTSGGTAALGCLVKDYFPEPVTVSWNSGALTSGVHTFPAVLQSSGLYSLSSVVTVPSSSLGTQTYICNVNHKPSNTKVDKKAEPKSCDKTHTCPPCPAPELLGGPSVFLFPPKPKDTLMISRTPEVTCVVVDVSHEDPEVKFNWYVDGVEVHNAKTKPREEQYNSTYRVVSVLTVLHQDWLNGKEYKCKVSNKALPAPIEKTISKAKGQPREPQVYTLPPSRDELTKNQVSLTCLVKGFYPSDIAVEWESNGQPENNYKTTPPVLDSDGSFFLYSKLTVDKSRWQQGNVFSCSVMHEALHNHYTQKSLSLSPGK

SEQ ID NO: 42 - protein, 214 aa, artificial sequence
  synthetic
DIQMTQSPSSLSASVGDRVTITCKASQDVWTDVAWYQQKPGKAPKLLIYWGSTRWTGVPSRFSGSGSGTDFTLTISSLQPEDFATYYCQQTNIYPLTFGGGTKVEIKRTVAAPSVFIFPPSDEQLKSGTASVVCLLNNFYPREAKVQWKVDNALQSGNSQESVTEQDSKDSTYSLSSTLTLSKADYEKHKVYACEVTHQGLSSPVTKSFNRGEC

SEQ ID NO: 43 - DNA, 351 bp, artificial sequence
  synthetic
gaagtgaagcttgaggagtctggaggaggcttggtgcaacctggaggatccatgaaactctcctgtgttgcctctggattcactttcagtaattattggatgaactgggtccgccagtctccagagaaggggcttgagtgggttgctgaaattagattgaaatctaataattatgcaacacattatgcggagtctgtgaaagggaggttcaccatctcaagagatgtttccaaaagtagtgtctacctgcaaatgaacaacttaagaactgaagacactggcatttattactgtaccgatacggccccgtttgcttactggggccaagggactctggtcactgtctctgca

SEQ ID NO: 44 - DNA, 321 bp, artificial sequence
  synthetic
gacattgtgatgacccagtctcacaaattcatgtccacatcagtaggagacagggtcagcatcacctgcaaggccagtcaggatgtgggtactgatgtagcctggtatcaacagaaaccagggcaatctcctaaactactgatttactgggcatccacccggcacactggagtccctgatcgcttcacaggcagtggatctgggacagatttcactctcaccattagcaatgtgcagtctgaagacttgtcagattatttctgtcagcaatatagcagctatcctctgacgttcggtggaggcaccaagctggaaatcaaa

SEQ ID NO: 45 - DNA, 351 bp, artificial sequence
  synthetic
gaagtgatgctggtggagtctggaggaggcttggtgcaacctggaggatccatgaaactctcctgtgttgcctctggattcactttcagtaattattggatgaactgggtccgccagtctccagagaaggggcttgagtgggttgctgaaattagattgaaatctaataattatgcaacacattatgcggagtctgtgaaagggaggttcaccatctcaagagatgtttccaaaagtggtgtctacctgcaaatgaacaacttaagaactgaagacactggcatttattactgtaccgatacggccccgtttgcttactggggccaagggactctggtcactgtctctgca

SEQ ID NO: 46 - DNA, 321 bp, artificial sequence
  synthetic
gacattgtgatgacccagtctcacaaattcttgtccacatcagtaggagccagggtcagcatcacctgcaaggccagtcaggatgtgggtactgatgtagcctggtatcaacagaaaccagggcaatctcctaaactactgatttactgggcatccacccggcacactggagtccctgatcgcttcacaggcagtggatctgggacagatttcactctcaccattagcaatgtgcagtctgaagacttgtccgattatttctgtcagcaatatagcagctatcctctgacgttcggtggaggcaccaagctggaaatcaaa

SEQ ID NO: 47 - DNA, 352 bp, artificial sequence
  synthetic
gaggtgatgctggtggagtctggaggaggcttggtgcaacctggaggatccatgaaactctcctgtgttgcctctggattcactttcagtaattattggatgaactgggtccgccagtctccagagaaggggcttgagtgggttgctgaaattagattgaaatctaataattatgcaacacattatgcggagtctgtgaaagggaggttcaccatctcaagagatgtttccaaaagtggtgtctacctgcaaatgaacaacttaagaactgaagacactggcatttattactgtaccgatacggccccgtttgcttactggggccaagggactctggtcactgtctctgcag

SEQ ID NO: 48 - DNA, 321 bp, artificial sequence
  synthetic
gatattgtgatgacccagactcccaaattcttgtccacatcagtaggagccagggtcagcatcacctgcaaggccagtcaggatgtgggtactgatgtagcctggtatcaacagaaaccagggcaatctcctaaactactgatttactgggcatccacccggcacactggagtccctgatcgcttcacaggcagtggatctgggacagatttcactctcaccattagcaatgtgcagtctgaagacttgtccgattatttctgtcagcaatatagcagctatcctctgacgttcggtggaggcaccaagctggaaatcaaa

SEQ ID NO: 49 - protein, 452 aa, artificial sequence
  synthetic
EVQLVESGGGLVQPGGSLRLSCAASGFTFSSYDIHWVRQATGKGLEWVSAIGPAGDTYYPGSVKGRFTISRENAKNSLYLQMNSLRAGDTAVYYCARGLITFGGLIAPFDYWGQGTLVTVSSASTKGPSVFPLAPSSKSTSGGTAALGCLVKDYFPEPVTVSWNSGALTSGVHTFPAVLQSSGLYSLSSVVTVPSSSLGTQTYICNVNHKPSNTKVDKKAEPKSCDKTHTCPPCPAPELLGGPSVFLFPPKPKDTLMISRTPEVTCVVVDVSHEDPEVKFNWYVDGVEVHNAKTKPREEQYNSTYRVVSVLTVLHQDWLNGKEYKCKVSNKALPAPIEKTISKAKGQPREPQVYTLPPSRDELTKNQVSLTCLVKGFYPSDIAVEWESNGQPENNYKTTPPVLDSDGSFFLYSKLTVDKSRWQQGNVFSCSVMHEALHNHYTQKSLSLSPGK

SEQ ID NO: 50 - protein, 214 aa, artificial sequence
  synthetic
EIVLTQSPGTLSLSPGERATLSCRASQSVSSTYLAWYQQKPGQAPRLLIYGASSRATGIPDRFSGSGSGTDFTLTISRLEPEDFAVYYCQHYDNSQTFGQGTKVEIKRTVAAPSVFIFPPSDEQLKSGTASVVCLLNNFYPREAKVQWKVDNALQSGNSQESVTEQDSKDSTYSLSSTLTLSKADYEKHKVYACEVTHQGLSSPVTKSFNRGEC

SEQ ID NO: 51 - protein, 478 aa, artificial sequence
  antigen Ang2
YNNFRKSMDSIGKKQYQVQHGSCSYTFLLPEMDNCRSSSSPYVSNAVQRDAPLEYDDSVQRLQVLENIMENNTQWLMKLENYIQDNMKKEMVEIQQNAVQNQTAVMIEIGTNLLNQTAEQTRKLTDVEAQVLNQTTRLELQLLEHSLSTNKLEKQILDQTSEINKLQDKNSFLEKKVLAMEDKHIIQLQSIKEEKDQLQVLVSKQNSIIEELEKKIVTATVNNSVLQKQQHDLMETVNNLLTMMSTSNSAKDPTVAKEEQISFRDCAEVFKSGHTTNGIYTLTFPNSTEEIKAYCDMEAGGGGWTIIQRREDGSVDFQRTWKEYKVGFGNPSGEYWLGNEFVSQLTNQQRYVLKIHLKDWEGNEAYSLYEHFYLSSEELNYRIHLKGLTGTAGKISSISQPGNDFSTKDGDNDKCICKCSQMLTGGWWFDACGPSNLNGMYYPQRQNTNKFNGIKWYYWKGSGYSLKATTMMIRPADF

SEQ ID NO: 52 - protein, 330 aa, artificial sequence
  antibody heavy chain constant region IgG
ASTKGPSVFPLAPSSKSTSGGTAALGCLVKDYFPEPVTVSWNSGALTSGVHTFPAVLQSSGLYSLSSVVTVPSSSLGTQTYICNVNHKPSNTKVDKKAEPKSCDKTHTCPPCPAPELLGGPSVFLFPPKPKDTLMISRTPEVTCVVVDVSHEDPEVKFNWYVDGVEVHNAKTKPREEQYNSTYRVVSVLTVLHQDWLNGKEYKCKVSNKALPAPIEKTISKAKGQPREPQVYTLPPSRDELTKNQVSLTCLVKGFYPSDIAVEWESNGQPENNYKTTPPVLDSDGSFFLYSKLTVDKSRWQQGNVFSCSVMHEALHNHYTQKSLSLSPGK

SEQ ID NO: 53 - protein, 107 aa, artificial sequence [sequence omitted]

SEQ ID NO: 54 - protein, 10 aa, artificial sequence
  synthetic
  misc_feature (5)..(7): Xaa can be any naturally occurring amino acid
  misc_feature (9)..(9): Xaa can be any naturally occurring amino acid
GFTFXXXWXN

SEQ ID NO: 55 - protein, 19 aa, artificial sequence
  synthetic
  misc_feature (8)..(8): Xaa can be any naturally occurring amino acid
  misc_feature (10)..(10): Xaa can be any naturally occurring amino acid
EIRLKSNXYXTHYAESVKG

SEQ ID NO: 56 - protein, 6 aa, artificial sequence
  synthetic
  misc_feature (2)..(2): Xaa can be any naturally occurring amino acid
  misc_feature (4)..(4): Xaa can be any naturally occurring amino acid
TXPXAY

SEQ ID NO: 57 - protein, 11 aa, artificial sequence
  synthetic
  misc_feature (5)..(5): Xaa can be any naturally occurring amino acid
  misc_feature (7)..(7): Xaa can be any naturally occurring amino acid
KASQXVXTDVA

SEQ ID NO: 58 - protein, 7 aa, artificial sequence
  synthetic
  misc_feature (2)..(2): Xaa can be any naturally occurring amino acid
  misc_feature (6)..(6): Xaa can be any naturally occurring amino acid
WXSTRXT

SEQ ID NO: 59 - protein, 9 aa, artificial sequence
  synthetic
  misc_feature (3)..(5): Xaa can be any naturally occurring amino acid
QQXXXYPLT

SEQ ID NO: 60 - protein, 434 aa, artificial sequence
  synthetic
PFVEMYSEIPEIIHMTEGRELVIPCRVTSPNITVTLKKFPLDTLIPDGKRIIWDSRKGFIISNATYKEIGLLTCEATVNGHLYKTNYLTHRQTVVLSPSHGIELSVGEKLVLNCTARTELNVGIDFNWEYPSSKHQHKKLVNRDLKTQSGSEMKKFLSTLTIDGVTRSDQGLYTCAASSGLMTKKNSTFVRVHEKGGGGGGGGGGGGDKTHTCPLCPAPELLGGPSVFLFPPKPKDTLMISRTPEVTCVVVDVSHEDPEVKFNWYVDGVEVHNAKTKPREEQYNSTYRVVSVLTVLHQDWLNGKEYKCKVSNKALPAPIEKTISKAKGQPREPQVYTLPPSRDELTKNQVSLTCLVKGFYPSDIAVEWESNGQPENNYKATPPVLDSDGSFFLYSKLTVDKSRWQQGNVFSCSVMHEALHNHYTQKSLSLSPGK